European Patent Application EP 4 520 840 A1, published March 12, 2025. Title: Suppression PCR-based selective enrichment sequencing. Applicant: Fraunhofer-Gesellschaft zur Förderung der angewandten Forschung e.V. Application EP. The sequence listing filed with the application follows.

SEQUENCE LISTING (41 sequences)

SEQ ID NO: 1 - DNA, 22 bp, synthetic construct
  source 1..22: mol_type = other DNA
tccgtcttagctgagtggcgta

SEQ ID NO: 2 - DNA, 19 bp, synthetic construct
  source 1..19: mol_type = other DNA
aagatgtggcgtgttacgg

SEQ ID NO: 3 - DNA, 17 bp, synthetic construct
  source 1..17: mol_type = other DNA
ggagacgaaacgttccg

SEQ ID NO: 4 - DNA, 17 bp, synthetic construct
  source 1..17: mol_type = other DNA
acatcgcttttggtggc

SEQ ID NO: 5 - DNA, 20 bp, synthetic construct
  source 1..20: mol_type = other DNA
aatcgatggtaaaggttggc

SEQ ID NO: 6 - DNA, 18 bp, synthetic construct
  source 1..18: mol_type = other DNA
gcattctgactggttgcc

SEQ ID NO: 7 - DNA, 18 bp, synthetic construct
  source 1..18: mol_type = other DNA
catcaccaggttcaaccc

SEQ ID NO: 8 - DNA, 19 bp, synthetic construct
  source 1..19: mol_type = other DNA
tgaggcacctatctcagcg

SEQ ID NO: 9 - DNA, 19 bp, synthetic construct
  source 1..19: mol_type = other DNA
gcacgtatgagcaagatgc

SEQ ID NO: 10 - DNA, 19 bp, synthetic construct
  source 1..19: mol_type = other DNA
tctgacaacaggcatgacg

SEQ ID NO: 11 - DNA, 18 bp, synthetic construct
  source 1..18: mol_type = other DNA
ccaataccgcacaaccga

SEQ ID NO: 12 - DNA, 19 bp, synthetic construct
  source 1..19: mol_type = other DNA
gaagtggatcaaatccggc

SEQ ID NO: 13 - DNA, 18 bp, synthetic construct
  source 1..18: mol_type = other DNA
caatgccaatctcagcgg

SEQ ID NO: 14 - DNA, 18 bp, synthetic construct
  source 1..18: mol_type = other DNA
aggcaagcaggatgtagc

SEQ ID NO: 15 - DNA, 22 bp, synthetic construct
  source 1..22: mol_type = other DNA
caaaggcttggaatactgagtg

SEQ ID NO: 16 - DNA, 19 bp, synthetic construct
  source 1..19: mol_type = other DNA
tcatatcgtcgagtggtgg

SEQ ID NO: 17 - DNA, 18 bp, synthetic construct
  source 1..18: mol_type = other DNA
gatcgagtcgttcatcgg

SEQ ID NO: 18 - DNA, 18 bp, synthetic construct
  source 1..18: mol_type = other DNA
caggatatcgctcaaccg

SEQ ID NO: 19 - DNA, 22 bp, synthetic construct
  source 1..22: mol_type = other DNA
gtaggtacatcatcgttaaggc

SEQ ID NO: 20 - DNA, 20 bp, synthetic construct
  source 1..20: mol_type = other DNA
gcgattattgttgctgaagg

SEQ ID NO: 21 - DNA, 19 bp, synthetic construct
  source 1..19: mol_type = other DNA
ggattgccttgtctaaccc

SEQ ID NO: 22 - DNA, 18 bp, synthetic construct
  source 1..18: mol_type = other DNA
ccatgaagtcggaatcgc

SEQ ID NO: 23 - DNA, 20 bp, synthetic construct
  source 1..20: mol_type = other DNA
gcaattgtagaaggcgtggc

SEQ ID NO: 24 - DNA, 19 bp, synthetic construct
  source 1..19: mol_type = other DNA
aagacgcactagcgaaagc

SEQ ID NO: 25 - DNA, 19 bp, synthetic construct
  source 1..19: mol_type = other DNA
gtggtggaagtctacaccg

SEQ ID NO: 26 - DNA, 20 bp, synthetic construct
  source 1..20: mol_type = other DNA
ggctatgggatgatattgcc

SEQ ID NO: 27 - DNA, 19 bp, synthetic construct
  source 1..19: mol_type = other DNA
tcggaaggagagaacatcc

SEQ ID NO: 28 - DNA, 21 bp, synthetic construct
  source 1..21: mol_type = other DNA
tctatagatggcaacacacgg

SEQ ID NO: 29 - DNA, 20 bp, synthetic construct
  source 1..20: mol_type = other DNA
gctatcgcaagttctaccgg

SEQ ID NO: 30 - DNA, 21 bp, synthetic construct
  source 1..21: mol_type = other DNA
ctgcctccatactttgtaggc

SEQ ID NO: 31 - DNA, 19 bp, synthetic construct
  source 1..19: mol_type = other DNA
ggtcgaaagcgtacttggc

SEQ ID NO: 32 - DNA, 20 bp, synthetic construct
  source 1..20: mol_type = other DNA
gcaactcgtagcaaataggc

SEQ ID NO: 33 - DNA, 16 bp, synthetic construct
  source 1..16: mol_type = other DNA
cagaaccgcgctaatt

SEQ ID NO: 34 - DNA, 15 bp, synthetic construct
  source 1..15: mol_type = other DNA
ctcgcgcgattatcc

SEQ ID NO: 35 - DNA, 19 bp, synthetic construct
  source 1..19: mol_type = other DNA
gaacatctgtggtatggcg

SEQ ID NO: 36 - DNA, 20 bp, synthetic construct
  source 1..20: mol_type = other DNA
gctatcgcaagttctaccgg

SEQ ID NO: 37 - DNA, 19 bp, synthetic construct
  source 1..19: mol_type = other DNA
agagcaggacagcaaggac

SEQ ID NO: 38 - DNA, 19 bp, synthetic construct
  source 1..19: mol_type = other DNA
gtcaatctggtctgcctca

SEQ ID NO: 39 - DNA, 43 bp, synthetic construct
  source 1..43: mol_type = other DNA
  modified_base 43: mod_base = OTHER; note = optional phosphothioate
tgtagcgtgaagacgacagaaagggcgtggtgcggagggcggt

SEQ ID NO: 40 - DNA, 12 bp, synthetic construct
  source 1..12: mol_type = other DNA
accgccctccgc

SEQ ID NO: 41 - DNA, 21 bp, synthetic construct
  source 1..21: mol_type = other DNA
tgtagcgtgaagacgacagaa